European Patent Application EP 4 183 889 A1, published May 24, 2023. Title: METHOD FOR THE IDENTIFICATION AND RAPID DETECTION OF BLUEFIN TUNA. Applicant: CONSEJO SUPERIOR DE INVESTIGACIONES CIENTÍFICAS INL - International Iberian Nanotechnology Laboratory. The sequence listing filed with the application follows.

SEQUENCE LISTING (14 sequences)

SEQ ID NO: 1 - DNA, 27 bp, Artificial Sequence
  Primer F2
tttacataaaccatacaaataaacctc

SEQ ID NO: 2 - DNA, 31 bp, Artificial Sequence
  Primer R3
ttacgagatgtcagagatgaggagacttggt

SEQ ID NO: 3 - DNA, 48 bp, Artificial Sequence
  Probe nfo RPA 2
tcatcttgaattcaggcgattaaacgagatttaagacctaacataaat

SEQ ID NO: 4 - DNA, 48 bp, Artificial Sequence
  Probe exo RPA 2
tacataaaccatacaaataaacctcaacattcatcttgaattcaggcg

SEQ ID NO: 5 - DNA, 34 bp, Artificial Sequence
  Primer F1
atgaagatttacataaaccatacaaataaacctc

SEQ ID NO: 6 - DNA, 28 bp, Artificial Sequence
  Primer F3
tttacataaaccatacaaataaacctca

SEQ ID NO: 7 - DNA, 34 bp, Artificial Sequence
  Primer R1
gtcagagatgaggagacttggtatggcttagacg

SEQ ID NO: 8 - DNA, 27 bp, Artificial Sequence
  Primer R2
gtcagagatgaggagacttggtatggc

SEQ ID NO: 9 - DNA, 48 bp, Artificial Sequence
  Probe nfo RPA 1
ttgaattcaggcgattaaacgagatttaagacctaacataaatctaaa

SEQ ID NO: 10 - DNA, 48 bp, Artificial Sequence
  Probe nfo RPA 3
ttcatcttgaattcaggcgattaaacgagatttaagacctaacataaa

SEQ ID NO: 11 - DNA, 48 bp, Artificial Sequence
  Probe exo RPA 1
ttacataaaccatacaaataaacctcaacattcatcttgaattcaggc

SEQ ID NO: 12 - DNA, 48 bp, Artificial Sequence
  Probe exo RPA 3
aaccatacaaataaacctcaacattcatcttgaattcaggcgattaaa

SEQ ID NO: 13 - DNA, 52 bp, Artificial Sequence
  Probe exo RPA 4
cttgaattcaggcgattaaacgagatttaagacctaacataaatctaaatcg

SEQ ID NO: 14 - DNA, 48 bp, Artificial Sequence
  Probe exo RPA 5
aattcaggcgattaaacgagatttaagacctaacataaatctaaatcg